European Patent Specification EP 3 504 325 B1, published July 3, 2024. Title: New paramyxovirus and uses thereof. Applicant: Universitaet Leipzig. The sequence listing filed with the application follows.

SEQUENCE LISTING (14 sequences)

SEQ ID NO: 1 - DNA, 16047 bp, Feline Paramyxovirus-Type 2
  complementary sequence of the genome of Feline Paramyxovirus-Type 2 (FPaV-2), Strain Gordon
accagacaaagatgtctgtgacctattctaacggttagattattacttgatatttaggaataacgattccattagtcaggtaagggagaggaatcagttattctataatggctagtttactcaggtcacttgcggcattcaagaaacacagagaacaaccaactgttccttctgggtcaggagggacgatcaaaggattaaaaaatacaattattgtgcctgttcctggagatacagtcatcactaccagatcgaacttactgttcagattagtctacataattggtaatccagatacacctttaagcacttcaacaggggcaataatatcattgttgacattatttgttgaatctccaggtcaattaattcaaagaatcgctgatgatcctgatgctgtttttaaattagtagaggtggttcctgaggttggtaatcctggagaattaacttttgcatctagaggaattaacttggataaacaagctcaacaatactttagattggctgagaaaaatgatcaaggatattatgtaagtttggggtttgaaaatccaccaaatgatgatgatataacgtcaagtcctgaaatctttaattatattttagcatctgtacttgcacagatctggattctcctagctaaggctgtaactgctccagacacagctgctgaggctgaaaaccgtaggtggattaaattgatgcaacaacgcagagtggatggtgagcttagattaagtaaaggatggttggacttagtgaggaataaaatcgcatcggatatcacaattagaaggtttatggtagcattagttcttgacattaaacgttctcctggaacaagaccaagaattgctgaaatgatttgtgatatagacaattatattgtggaggccggactggcaagttttctgttaactatcaaatttggtatagaaacacgttacccggcattagcgttacatgagttttcgggggaattagccactattgaaggactcatgaaattgtaccagtctatgggagaaatggcaccatacatggtcattctagagaattcgatccagactaggtttagtgctgggtcttatccgttactctggagctatgctatgggtgttggtgtagaacttgaaagatcaatgagtggattaaacttcacaagaagtttctttgatcctacgtacttcaggttgggtcaggagatggtaagaaggtcttcaggaatggttaatagctcatttgccaaagaacttggactatctgaacatgaaacacaacttgttagccagatcattaactcaggtggtgagtcaggtataccgaaatttgatggatttagagcaaacccaacaacatttctaggggctaaggacaacatcactgataggagtgaagatccattgattgcaattccagggtcatcaggacaaccattgccaggttatgaccccaatatctcaggtgactcatatagaattgatagtagcactaaagacacaaacaatatatcagatggaggaacaaatccaagtcatgatgtttccaattctgctatggaagagctgagaagattggtagagtctaccaacaagattgatacaaagaaatctgaaagcccaggcatcgttaatcattacaacgatactgaccttctgagataataaggatatattcaggtagatctttacagaatttaaattaagaaaaacttaggacctcaaggttcacactcctctggcctttatcagaattcggccaattcctcactcactccatgtcagcagaacaaatccaacaagttagacatggccttgaatccttgcaagagatcaaaaacaaccctccaccctctcaagatgtcaatcttgccagggaaatttacgaatccattaaacaaacaggaacaccttcaacacaaggagggaccattacaggaaataatactgcgtcagggtgtgacaattactcaatgcatagccagggatcaggtccttctgtttcaggtgctgacaagaatatcgagagacttactggacccgattattcagaattatgggatccagaaggtaacctctgcatgctattcgaaagcgatgatgatgacaacaattattcagagattaatggccggtctaccgctatcgaaggattggatgaacagaataataaggacccaggtattaaacaatcaggagatcagtgttctgaaggagtgtctaagattaattcatcttctagtccccaagaagctacattatcttctgggagatctgatatatctgggacaggagtatctccctgtgcctctttggatataactgttaatgaattagaagatgcaactgttaagaatagtaataatatgaaaggaaattggccaatcccaaagttgcttgtcaaaccaccaccaagaatgaaatcactttctgactctgttacaccattaaaaggggccaccgacgggaaatcagtcttacctgggatggagattacattgtccgggaagaatggtgcaaccctacctgtacacccatttacacaacctataaaagactcaaatgcagatgtaagcaatgtccgtcaacatgtcccaagtgtgactgatggtcatagtgatgataatgaggaagtacccggtttgcataaagaaactatagacaaagctgatctatctatgcaggacatatacaatttaattcttggatttaaggatgattacaggaaactatcaaataaattggatatgatactagagatgaaacaagatattgataatcttaaaaagagtagtgcaaaaatacaacttgcattatcaacaattgaaggacatctgtccagtgttatgattgctattccaggttcaggtattgatataaatcaagatgagaagaaggatcaattaaactctgacttaaagccattactagggagggaccattgccgtgcatttcgtgaagtcactaatcctttagatgaaacgtcattgaccaacgctccgaccaaacatgttgctaagatcaacaaaaattgcactcttcagaaaatcaataacaatgagacatctgcaattaagtttgtacctaatgatagccatgcaagtatctcgactatcaagtctattgtcaaatcctcaaaccttaatcaagagcttaaagtcaagttactgacaattctatctcaaattaaaggggtagacaatattaaggagttttatgagaaagttatgatattgatcaagaataataactgatcttgactaatcaatagatactacttatcaaatctcgctctgacatcaagtgaattcatctttattaacaagtattaatcttaaataattataaaaaacttaggagttcaggattagtgggtcatatacaatatgactgagatattcaatctggatgaaagttcatggtcagtcaagggaacactggacccattgacgcctgatacttatcctgatgggcgcctagtacccaagattcgggttattgatcccggtctaggtgatcgtaaaagtggaggatatatgtacttactccttcacggtgtcatcgaggacagtgagaccgtcataaatccgaaagggagagcatttggagctttccctttaggcgtagggcaatcaaccgagaacccagaagacttatttaaggaaatattaaccctcaacattgttactcgcaggactgctggcttcaatgaaaaattggtgtattataatactacacctctaaatctactaaccccttggaaaaaagtactagcatatggaagtatctttactgctaatcaggtctgcaataatacaagttctatccctatagacattcctcagaaatttcgacctgtctatttaactgttaccaagttatcggatgatggatattatcagatacctaaaatgatacaggatttcaaatcatcaaactctgttgcatttaacatccttgtgcatctatcaatgggaacaattttacttgactcatctaaaggctctcgagtaggaaaccctgcagaaaatttgatcacattcatgattcatattgggaatttcaaacggaagaataataaagcttattctcccgaatattgtaagaggaaaataatgaggcttggattaattttctcactaggagccattggtggaacaagtttgcatattcgatgcacaggcaaaatgagtaagagattacaagcctacttagggtttaaaagaactttatgttatcctctgatgtatgtcaatgagggtctaaataaaaccttatggagaaatgaatgcaaaattgagaaggttcaagcagtattacagccatcagttccgaatgaatttaagatttatgatgatataatcattgataacacgaatggcctctttaaggttaagtaagctgtgactagtatcaggagttactagtcaaaatcatgtgttgatatccgaattaatagctttaagttgaatatattaaacctgtgataatttaaatttgaaacataattagtatgtagtattgtattaatcagtttataatcttgtttgaggatccaaattataaccctattaggtattgccactccagtcttacaggtaaatctaagcgaatatacaaataattgatattcgggattaaacaatacttgtatattaatccataggtatattagattttactatattcaattattataatgtttattgagttaagctctcatgattataaaaaactaaggattccacataatcacagtttgattgccaattgatgtgtttagtattagttgtgtgaaatattgatattaataaggttaatcaacttttgtacagaagtgaaagtgtaattagatagaaatagattaatccttagtagccgttttgataattgaattgattcttgttttaattctgaattgagattattaatcaccagctcggcataatgtataagattaaggttgtaatcatgggttttttactgttatcagatattacatttgcacaggtaggttgggataatttaacctcaattggagttataagtactaaacaatataactataagataactactttgaatactaatcaactcatggtgatcaaaatggtacccaatatatcatcaattattaactgtactaaacttgaattagcaaaatatagggaactgattacaggaatactgagaccaattaatgaatcattagaattgatgaattcatatatcaacatgagaacaggttcagagagattcataggggctgttatagcaggagtagctctaggggttgcaactgcggcgcagataacatcgggaattgccttacataattcgattatgaataaaaaacagatacaggaattaaggaaagcccttagtactacaaataaggcaattgatgagataaggattgcaggtgaaagaactctgatagctgtccaaggtgtgcaagattacattaacaatgttattatccctatgcaagagaaactccagtgcgatattttagcctcacagctatctattgccctactcagatactatactaatatactgactgtttttggaccaagtataagagatcctattactagtacaatttctatacaagctctcagtcaagcattcaatggtaatctacaggcattgcttgatggattagggtatactggacaagacttacatgatctcatagaaagtagatctatcactggtcaaattattcacgctgatatgactgatttattccttgtattgagaatcaattatccatctattacggatatgcaaggagtggtaatatatgagctgaattctatcacatatcatattggacctgaagagtggtacactattatgcctaatttcatagctgttcagggatttctggtatctaatttcgatgaacgtaaatgttcaattactaaaacaagtatactgtgtcaacagaattcaatttatcctatgtcaaccgaaatgcaaagatgtataaaaggtgagattaaattctgtccaaggtccaaagcaattgggacattagttaatcgatttatattaattaatgggaatctaatggccaattgtttgggtattatctgtagatgttatacctcaggtcaaattataacgcaagacccaaataaattaatcacaattatatcacaagaagaatgtagagaggttggtgttgatgggattcgtataatggtggggcctaaaaaattaccggatgttatctttaatgccagactagaaataggtgtacctatctcattaagcaagctggatgttgggaccgacttggcaattgcttcagctaaactcaataactctaaggcacttttggagcagtctgataaaatcttaaattctatgtctaagttggattctttaaattcacgtatcttaggatctgtctttataattatgataatcttcgtgactgtaattgtgattatttggattatttgtaaaaagtgtagaaataagaggaacaaattaagtgcttctattgaacccctctacatacctccctcttataattcaccccatagcatagttaaatctatttgaaatataagtgtataatctgatataacagatgcagtagaattattaatcaatgataatattattatgataatgattcagttagatgttcattgtatctcataacttaatattgacaaatttcaattagttaaatttattctcttcataatatgtatttgtttaattatcctagattcatgtactgttattaaattggtcatctttaataactaactcagcaatactatcctatacacatgtattagctaataacgatgtaatattgccatttaataataagtacctagtagaatgggaagcattagctgtagtcaatgaaccattacctgctcaattagaaaaaacttaggaatccatgttaatgggagctggccatcatggaatctaataacaacaagtactataaagattcaaaccggtattttagcaagatactagatgagaacaagacggtaaataatcatctgtatagtcttagtataaggataattaccgttatagctattgttgtgagtctaattgcaacaacaataaccatcattaatgctataagcggaaggactactcttaataataatatggacatgctactcaaccaacaagacaagattaataatatcaaggaaatgatatttgatcgtatctatcccctgataaatgccatgagtacagagcttggtcttcacattccaactttattggatgagctgactaaatcaattgatcaaaaaatcaagataatgactccaccacttgaaactacaacatctaatctcaattggtgtatcaaccccccaaatggcattattgtagatcctaaaggttattgtgaaggcttggaactgtcaaaaacttataagttattacttgatcaattagatatgttaagaaagaaatcacttattattaataagaaaagtattaatcagtgtagacttgttgatagttcgaatatcgtctttgcaacagttaatatacaatctacaccgagattcttaaatcttggtcacacagttagtaaccaacgtataacattcggtcaaggaacatatagtagcacttatattataactatacaagaggatggattaactgatgttcagtaccgagtatttgaaataggatatatctcagatcaatttggaaccttcccttctctaatcgtttccagagtactacctgtgcgaatggtacttggaatggaatcttgtacactgaccagtgacaagtttgggggttattttttatgcatgaacattccgacacgctctatatatgattatgtcaacataagagacttaaagtcactatacgtcacaatccctcattatggcaaaattaattacacttactttaattttgggaaagtcagaagcccacatgaaattgataagatttggcttacatcagaaaggggacagatgatttcaggttactttgcagcatttgttacgattacaattagaaattataacaattatccctataaatgcttacataacccgtgtcttgaaagatctgagagttattgcaaaggatggtacaaaaatattacaggtactgatgatgttccaatattagcatatctattagttgaaatgaatgatgaggaaggacccttaattacattggttgagataccaccttacaattatacggctccttctcataattccctttactatgatgataaaattaacaaattaataatgacaacatctcatataggatacattcaaatcaatgaagtgcatgaagtcattgtcggggataatcttaaggctattctcttaaacagattatctgatgaacaccctactcttactgcttgtagatttaatcaggaaattaaagagcgacatatatctgatggattaataatatctaactctgctcttattgatatacaagaacgtatgtatgttacagttaaggctgttccacccataggaaattataacttcacggtagagttgcattcacggtcaaatacatcttacgtagggttgccaaggcagttcaatgctaggtatgacaaactgcatctcgaatgctttgcctgggataggtcttggtggtgcgctttgatacctcaattttcattaagttggaatgaatctctttcagtagatactgccattttcaacttaataaactgtaattaagtttgtggcttgttctagattgatcatttgaataacagttgattaagccaaagttagtaaatacatacattaacctgttcttgaccaagtatatatcccaatccaattataaaaaacttaggactcaaggtgttgatggcaatggagcaatcagattatcaagatattttatatccagaggtacatctcaacagtcctatagttatctctaaattagtgggtattttggagtattctaaggttgttcacaatcagcagttatctgatcacacaatagtcaagaatatacaatttagattgagaaatggattcaatagtccaagaatacaaacactgttagttatgggtgaaattatcaataaaatcaaaaataaatacccaaattatttgcacataccttatcctgaatgtaatcaaaagttatttaggatagctgacccggagttaacatctaaactagaagccctcttggacaaaggtgacacattatatcttaagattaagacagagatcatagcttgtttcgataagttaaaaactaaaatgagcataaccaatgatctgattagtgacaataggcagctaatttcagatctacctataattgtcaagggatctcaatggtttttcccttttttgctctggttctctgttaaaactgagactaggaactgtattcgacaaaatcaaaaaactcgtgttaggtcacaataccgacctcatttgtcagaaactaaaagaattacgctggtcgttactcatgacttgatcacaatatttgaccacgtcaacaaatgtatatatcatctgacttttgagatgttgttgatgtattgtgatgtagtagaagggaggttaatgaccgaagcatctatgagtctagatcacagatttattaacctattgtcgagggtccagtatatgtgggatctattagatgggatgtttgagagtctaggaaatcagctatattcaatcattgcactcttagaacctctctctcttgcctatctacagttgatggatgcagacccacagatacggggtacatttttacaccattgcctttcagagttggaagaactcttatttagtaaattcccttttgatcctgtaatttatgaaaatctaattagtggacttgattacatctatttaacagacgatattcatttaactgctgagatattttctttctttagaagttttggtcatccttatttagaagcacaaaatgcagctagcaatgttaggaaatatatgaatcaacctaaagttatctcataccagactctaatgcaaggacatgcaattttttgtggcattataataaatgggttcagagatcgtcacggagggacatggccacccgtagagctaccacatcatgcatccgctgtaattagaaatgctcagttatctggagaaggattaacacctgagcagtgtgctcaatactggaggtcattttgtggatttaaatttaaatgttttatgccattaagtttagatagcgacctcaccatgtaccttagagacaaggcattatcacctattaagaatgagtgggactctgtgtatgctaaagagtatttaagatacaaccctggcttaccgactagctctcgaagattagtcaatgtatttcttgaagatgataaatttgatccgtacgaaatgattatgtacgtaataaacggtgattatttaagggataatgagttcaatctctcatatagtcttaaagaaaaggagatcaaggaggtaggccgattgttcgctaaaatgacttataaaatgagagcttgtcaggtaatagcagaaaatttaattgcaaatggagttgggaaattttttaaagacaatgggatggcgaaggatgaacataaattaaccaaaacattacataagctggccatttctggtgtacctaaagataattttcaactctatttaagtgaatgttgggaacaagtggtagaacaatgcgtaaccagtacgcaaacaaaaaatcaaattatcagttcacactcaagaaaatcagttgcatcaaagtttccaagatcaaatcccaatgataggggtattctaaatagtggcagacatttgaataaacatccaaaacatccttcaaacaccgaatactatgaaactgtcagtagttttataactactgatctcaagaaatattgcctcaactggcgctatgaatcaagtagtgtgtttgcagaaagactcaatgagatttatgggttaccaggattttttcattggcttcatagaattttggagaaatctgtattatatgttagtgatccatccagtccacctgattttgatcaacatgttgatattgattcagttccaaatgatcatatttttatcaaatacccaatgggtgggatagaaggattttgtcaaaaattatggacaatcagcacaatcccatttttatatttagcagcttttgatacaggggttagaatatcttcgttggttcaaggtgataatcaagcaattgcagtgaccaaaagagttccatcgtcctggagttattcgagaaaaaaagaggagtcaactaaagttacaacacaatattttttaaacttaagacaacgcttacatgatataggtcatgagttaaaggcaaatgagactattatatcttcacacttttttgtttactctaagggtatttattatgatggtatacttctttcacaatcccttaaaagtattgcaagatgtgttttttggtccgagacaattgtcgatgagactaggtcagcttgcagcaatatatccactacccttgctaaagctattgaacggggttatgataaattcgtggcatacgctattaatatatataagactatacaccaggtcttaattgcattatcttttactattaatcccactatgactccggacataacagaacctttttataaaagtttagatttacttaaaaacctcattctgataccagcaccattgggtgggatgaattacatgaatatgagcagattatttgttagaaacataggtgatcccattacagcttcatttgctgacatcaagcgtatgatcgaatgcgggttattagggcacaatgttctctcacaaataatgtatcagaaatgtggtacctcgaaatacttagattgggctagtgacccttattccataaatcttccttatagtcaaagcatgaccaaagtattaaaaaatataaccgcgagatatgttctcatgcacagtcctaaccctatgctaaaagatttattccatgagaagtcacaagaagaagatgagattcttgctgaatttttgctggatcgtcagttaataatccctagagctgcacatgaaattttatcgaattcagtaacaggagctagagagtcgattgcagggatgcttgatactactaaaggacttattcgagccagtatgtcaagaggtggtctgacatcttcacttgtgttgaaattgtcaacatatgattatcaacaatttagaacatgccttgaatggctttatgcccctaccacaggaatagcagtaagtgctgattcttgttcagtttttttagccagagctattcgaaaaaggatgtgggttcacctgactaaaggaagagaaatttatggcctagaagtgcctgatatattagaatgtatgcagagcaatgtaattgttgatcatgaagattgttattcatgtattcaaggatcaagatactacacatggttttttgtaccttctaattgtcagcttgatcagattaacaagtctacaaattctctacgggttccttacattggctctactacagaggaaagaagtgacatgaaattatcatacgtcagatcccctagtaggccacttaaggcagcagtccgaattgcagcagtctacacatgggcatacggtgatgacgatctgtcttggcgtgaggcttggtacttggcaaggactagggcaaatgttactttcgatgagcttaaattagtaacacccatagctacctctacgaacttggcacatagattaagggacaggagtactcaagttaagtattcaggaacttcattagtaagagtggcacgctatacaacaatatccaatgataatatgtcatttgtcattaatgacaaaaaggtagatactaattttgtctatcaacagggcatgttattgggtttgagtatcctagaatatatatttagatactgtaaaagtactggtcaatcaaatactgtagttcacttgcatgcagatgttaattgttgcataatccaaatgacagatcaaccttatactccaagcttaacgaaaaaattacctgagattaaacctattaataataagttgatttatgatccagctcctataattgatactgatgcagctaggttatattctcagaagtacttatcacacctgatagattttccaaattggtcaatgaatcagctaaatgtagttttagcaaaagtagttgcaatatctattgtggacttgataactaaagcgagtaaagatcatctcaatgaaattatggcagttgttggagatgatgacattaatagctttataacagaatttttgctagttgatccgaggctatttacattgtacttaggtcaatacacgtcacttcaatgggcatatgaaattcattatcaccgacccgtaggcaaataccagatggcagaagtgttacacactttactgtcaagagcaagtaaaggtatatttaatatattaactaatgcttttagtcatcctagagtttacaaaagattttgggaatgtggattactggagcctatttatggaccatacatagggagccaaaatttatatagtacagtaattgattacctttacaatgcttatataacttatttagatgcttatctatctgatcatatcgaagatgcagacatagtaatatgtgagacagaagaaacttgtctagctaataggattgataactatcaaggtaggcatctagccgtacttattgatctttattgtgattctactaggtgtcctaatataaaagggtcagacacaatcatgcgaaactcaattctcaaatcttttattgataatgagagaaggacaagtccattaggtctaacatggaatcttgatccattactcatagatcatttcagttgttcaattacttatctgaggagaggtattattaaacagattaggctaaggtttgatccaaacatatctattgagttggttaaattggcaaaacctgaagtgattcatcaaggaccaaaaataccgtcttcttgggcccttatagatattaatcctgaggtcaatgatcttaatacagttttcggagaattaaatagtaaatggaaagatattcctattggacaaattagaattcaaaattatgagatccatgcttaccgaagaattggagttaattcaactgcatgttataaagcattggaaatgctatctgtactaacccggtttatgtctaacccagcaggagctttgtttttaggagagggtgcagggtcaatgttagttacctatcgtgcgtttatcccgttcaagagaatttattataatagtggaatttctatacaaaatattcaaagccaaagagaactaagtctatacccatctgaagtagccttggttgataataaaaatcgtttgaccagtgatcctgatatcaaagtcttatttaatggcaagccagaatccacgtgggttgggaatatagactgctttgcttatattctgagtcatattgaaacttctagtttaacattaatccacagtgatattgaatctagcttgagtaaaacaaagaataagattcttgaggagctttgccatattctatcaatggcactgattttaggaaagattggatctgtattagttattaagctgttaccacgggttggtgactacacatattcattttgcaagtatgcgtcagaattctaccaacagaatttttttattttacctagatttagcaacatgtcatcatctgaaatttactacgttggagttcatttaaataccaatagactggttgatccagataggattgtgcaatatataatcaggaatctccaatctactccagttactttcttatcttacattttggaaactaaatatagaaataatatggttacaaattatgggctctgcttgtctgatggacataaaagcgattacttgtcatcaatcaccaagatagaaaatgttcttttatcatgtggattggaattgaatggacctaagattatacagcaattatctggacatgactacgccaatggagagattagcttagaatcaagtataatggtactggttagagaatatctaaatgcaactatccaaggtcgggaaacactaggtcttttttcaccttaccctgtgttacatgagagtcagttaagagaaattaacaggtgcattgcattgaagtatgttgtatatttacttttttactcaacctctgtaggatctagtagacaaatcatgagcaatctcagaaaaggagtattaatgtatgacttaagagatgagtttttcatggaaaggttatcaacaaatttcaagaaaaaaataatgtcacaagaggttaaaactacatggatctttaatattgatgtaccaacaagaaaagctctgtataaattagttggttattcacttatcattaatcacgtataacaagtgtattgagttggtaatattctagatgaacaagtataggtttatgtacagtaagtgattaaatattagattcaggtagataaacttcctaatagtgtatcctatagataacctaaggctatttaatgttagattaattagaaaaaacttcttgaattatgatagacttcaacccctggctaagacttatcatttaaaattataaccaagttgtcctgataatatcagatctcattaattacttgatagcgtaatataacaggtgcatgatgatcctttattactcatatacctgttattaagctcctgttcaaattatcccctatttaagttgccttttaaattacctaatatgttttgtaatgagaaacattgatacatacaaagctaaagaagcctgattttatctaaggttgtatctaattgttgtcaatttataattcggaatatctgggccctaaacctcctccaaatatactaaaaggttttaaaaaaacaaaaaaggtttcttacttattgtacggacctatagctttcttttgtctggt

SEQ ID NO: 2 - protein, 519 aa, Feline Paramyxovirus-Type 2
  Nucleocapsid protein, Strain Gordon
MASLLRSLAAFKKHREQPTVPSGSGGTIKGLKNTIIVPVPGDTVITTRSNLLFRLVYIIGNPDTPLSTSTGAIISLLTLFVESPGQLIQRIADDPDAVFKLVEVVPEVGNPGELTFASRGINLDKQAQQYFRLAEKNDQGYYVSLGFENPPNDDDITSSPEIFNYILASVLAQIWILLAKAVTAPDTAAEAENRRWIKLMQQRRVDGELRLSKGWLDLVRNKIASDITIRRFMVALVLDIKRSPGTRPRIAEMICDIDNYIVEAGLASFLLTIKFGIETRYPALALHEFSGELATIEGLMKLYQSMGEMAPYMVILENSIQTRFSAGSYPLLWSYAMGVGVELERSMSGLNFTRSFFDPTYFRLGQEMVRRSSGMVNSSFAKELGLSEHETQLVSQIINSGGESGIPKFDGFRANPTTFLGAKDNITDRSEDPLIAIPGSSGQPLPGYDPNISGDSYRIDSSTKDTNNISDGGTNPSHDVSNSAMEELRRLVESTNKIDTKKSESPGIVNHYNDTDLLR

SEQ ID NO: 3 - protein, 491 aa, Feline Paramyxovirus-Type 2
  Phosphoprotein, Strain Gordon
MSAEQIQQVRHGLESLQEIKNNPPPSQDVNLAREIYESIKQTGTPSTQGGTITGNNTASGCDNYSMHSQGSGPSVSGADKNIERLTGPDYSELWDPEGNLCMLFESDDDDNNYSEINGRSTAIEGLDEQNNKDPGIKQSGDQCSEGVSKINSSSSPQEATLSSGRSDISGTGVSPCASLDITVNELEDATVKNSNNMKGNWPIPKLLVKPPPRMKSLSDSVTPLKGATDGKSVLPGMEITLSGKNGATLPVHPFTQPIKDSNADVSNVRQHVPSVTDGHSDDNEEVPGLHKETIDKADLSMQDIYNLILGFKDDYRKLSNKLDMILEMKQDIDNLKKSSAKIQLALSTIEGHLSSVMIAIPGSGIDINQDEKKDQLNSDLKPLLGRDHCRAFREVTNPLDETSLTNAPTKHVAKINKNCTLQKINNNETSAIKFVPNDSHASISTIKSIVKSSNLNQELKVKLLTILSQIKGVDNIKEFYEKVMILIKNNN

SEQ ID NO: 4 - protein, 337 aa, Feline Paramyxovirus-Type 2
  Matrix protein, Strain Gordon
MTEIFNLDESSWSVKGTLDPLTPDTYPDGRLVPKIRVIDPGLGDRKSGGYMYLLLHGVIEDSETVINPKGRAFGAFPLGVGQSTENPEDLFKEILTLNIVTRRTAGFNEKLVYYNTTPLNLLTPWKKVLAYGSIFTANQVCNNTSSIPIDIPQKFRPVYLTVTKLSDDGYYQIPKMIQDFKSSNSVAFNILVHLSMGTILLDSSKGSRVGNPAENLITFMIHIGNFKRKNNKAYSPEYCKRKIMRLGLIFSLGAIGGTSLHIRCTGKMSKRLQAYLGFKRTLCYPLMYVNEGLNKTLWRNECKIEKVQAVLQPSVPNEFKIYDDIIIDNTNGLFKVK

SEQ ID NO: 5 - protein, 541 aa, Feline Paramyxovirus-Type 2
  Fusion protein, Strain Gordon
MYKIKVVIMGFLLLSDITFAQVGWDNLTSIGVISTKQYNYKITTLNTNQLMVIKMVPNISSIINCTKLELAKYRELITGILRPINESLELMNSYINMRTGSERFIGAVIAGVALGVATAAQITSGIALHNSIMNKKQIQELRKALSTTNKAIDEIRIAGERTLIAVQGVQDYINNVIIPMQEKLQCDILASQLSIALLRYYTNILTVFGPSIRDPITSTISIQALSQAFNGNLQALLDGLGYTGQDLHDLIESRSITGQIIHADMTDLFLVLRINYPSITDMQGVVIYELNSITYHIGPEEWYTIMPNFIAVQGFLVSNFDERKCSITKTSILCQQNSIYPMSTEMQRCIKGEIKFCPRSKAIGTLVNRFILINGNLMANCLGIICRCYTSGQIITQDPNKLITIISQEECREVGVDGIRIMVGPKKLPDVIFNARLEIGVPISLSKLDVGTDLAIASAKLNNSKALLEQSDKILNSMSKLDSLNSRILGSVFIIMIIFVTVIVIIWIICKKCRNKRNKLSASIEPLYIPPSYNSPHSIVK

SEQ ID NO: 6 - protein, 595 aa, Feline Paramyxovirus-Type 2
  Hemagglutinin, Strain Gordon
MESNNNKYYKDSNRYFSKILDENKTVNNHLYSLSIRIITVIAIVVSLIATTITIINAISGRTTLNNNMDMLLNQQDKINNIKEMIFDRIYPLINAMSTELGLHIPTLLDELTKSIDQKIKIMTPPLETTTSNLNWCINPPNGIIVDPKGYCEGLELSKTYKLLLDQLDMLRKKSLIINKKSINQCRLVDSSNIVFATVNIQSTPRFLNLGHTVSNQRITFGQGTYSSTYIITIQEDGLTDVQYRVFEIGYISDQFGTFPSLIVSRVLPVRMVLGMESCTLTSDKFGGYFLCMNIPTRSIYDYVNIRDLKSLYVTIPHYGKINYTYFNFGKVRSPHEIDKIWLTSERGQMISGYFAAFVTITIRNYNNYPYKCLHNPCLERSESYCKGWYKNITGTDDVPILAYLLVEMNDEEGPLITLVEIPPYNYTAPSHNSLYYDDKINKLIMTTSHIGYIQINEVHEVIVGDNLKAILLNRLSDEHPTLTACRFNQEIKERHISDGLIISNSALIDIQERMYVTVKAVPPIGNYNFTVELHSRSNTSYVGLPRQFNARYDKLHLECFAWDRSWWCALIPQFSLSWNESLSVDTAIFNLINCN

SEQ ID NO: 7 - protein, 2202 aa, Feline Paramyxovirus-Type 2
  Polymerase, Strain Gordon
MEQSDYQDILYPEVHLNSPIVISKLVGILEYSKVVHNQQLSDHTIVKNIQFRLRNGFNSPRIQTLLVMGEIINKIKNKYPNYLHIPYPECNQKLFRIADPELTSKLEALLDKGDTLYLKIKTEIIACFDKLKTKMSITNDLISDNRQLISDLPIIVKGSQWFFPFLLWFSVKTETRNCIRQNQKTRVRSQYRPHLSETKRITLVVTHDLITIFDHVNKCIYHLTFEMLLMYCDVVEGRLMTEASMSLDHRFINLLSRVQYMWDLLDGMFESLGNQLYSIIALLEPLSLAYLQLMDADPQIRGTFLHHCLSELEELLFSKFPFDPVIYENLISGLDYIYLTDDIHLTAEIFSFFRSFGHPYLEAQNAASNVRKYMNQPKVISYQTLMQGHAIFCGIIINGFRDRHGGTWPPVELPHHASAVIRNAQLSGEGLTPEQCAQYWRSFCGFKFKCFMPLSLDSDLTMYLRDKALSPIKNEWDSVYAKEYLRYNPGLPTSSRRLVNVFLEDDKFDPYEMIMYVINGDYLRDNEFNLSYSLKEKEIKEVGRLFAKMTYKMRACQVIAENLIANGVGKFFKDNGMAKDEHKLTKTLHKLAISGVPKDNFQLYLSECWEQVVEQCVTSTQTKNQIISSHSRKSVASKFPRSNPNDRGILNSGRHLNKHPKHPSNTEYYETVSSFITTDLKKYCLNWRYESSSVFAERLNEIYGLPGFFHWLHRILEKSVLYVSDPSSPPDFDQHVDIDSVPNDHIFIKYPMGGIEGFCQKLWTISTIPFLYLAAFDTGVRISSLVQGDNQAIAVTKRVPSSWSYSRKKEESTKVTTQYFLNLRQRLHDIGHELKANETIISSHFFVYSKGIYYDGILLSQSLKSIARCVFWSETIVDETRSACSNISTTLAKAIERGYDKFVAYAINIYKTIHQVLIALSFTINPTMTPDITEPFYKSLDLLKNLILIPAPLGGMNYMNMSRLFVRNIGDPITASFADIKRMIECGLLGHNVLSQIMYQKCGTSKYLDWASDPYSINLPYSQSMTKVLKNITARYVLMHSPNPMLKDLFHEKSQEEDEILAEFLLDRQLIIPRAAHEILSNSVTGARESIAGMLDTTKGLIRASMSRGGLTSSLVLKLSTYDYQQFRTCLEWLYAPTTGIAVSADSCSVFLARAIRKRMWVHLTKGREIYGLEVPDILECMQSNVIVDHEDCYSCIQGSRYYTWFFVPSNCQLDQINKSTNSLRVPYIGSTTEERSDMKLSYVRSPSRPLKAAVRIAAVYTWAYGDDDLSWREAWYLARTRANVTFDELKLVTPIATSTNLAHRLRDRSTQVKYSGTSLVRVARYTTISNDNMSFVINDKKVDTNFVYQQGMLLGLSILEYIFRYCKSTGQSNTVVHLHADVNCCIIQMTDQPYTPSLTKKLPEIKPINNKLIYDPAPIIDTDAARLYSQKYLSHLIDFPNWSMNQLNVVLAKVVAISIVDLITKASKDHLNEIMAVVGDDDINSFITEFLLVDPRLFTLYLGQYTSLQWAYEIHYHRPVGKYQMAEVLHTLLSRASKGIFNILTNAFSHPRVYKRFWECGLLEPIYGPYIGSQNLYSTVIDYLYNAYITYLDAYLSDHIEDADIVICETEETCLANRIDNYQGRHLAVLIDLYCDSTRCPNIKGSDTIMRNSILKSFIDNERRTSPLGLTWNLDPLLIDHFSCSITYLRRGIIKQIRLRFDPNISIELVKLAKPEVIHQGPKIPSSWALIDINPEVNDLNTVFGELNSKWKDIPIGQIRIQNYEIHAYRRIGVNSTACYKALEMLSVLTRFMSNPAGALFLGEGAGSMLVTYRAFIPFKRIYYNSGISIQNIQSQRELSLYPSEVALVDNKNRLTSDPDIKVLFNGKPESTWVGNIDCFAYILSHIETSSLTLIHSDIESSLSKTKNKILEELCHILSMALILGKIGSVLVIKLLPRVGDYTYSFCKYASEFYQQNFFILPRFSNMSSSEIYYVGVHLNTNRLVDPDRIVQYIIRNLQSTPVTFLSYILETKYRNNMVTNYGLCLSDGHKSDYLSSITKIENVLLSCGLELNGPKIIQQLSGHDYANGEISLESSIMVLVREYLNATIQGRETLGLFSPYPVLHESQLREINRCIALKYVVYLLFYSTSVGSSRQIMSNLRKGVLMYDLRDEFFMERLSTNFKKKIMSQEVKTTWIFNIDVPTRKALYKLVGYSLIINHV

SEQ ID NO: 8 - DNA, 16045 bp, Feline Paramyxovirus-Type 2
  complementary sequence of the genome of Feline Paramyxovirus-Type 2 (FPaV-2), Strain TV25
accagacaaagatgtctgtgacctattctaacggttagattattacttgatatttaggaataacgattccattagtcaggtaagggagaggaatcagttattctataatggctagtttactcaggtcacttgcggcattcaagaaacacagagaacaaccaactgttccttctgggtcaggagggacgatcaaaggattaaaaaatacaattattgtgcctgttcctggagatacagtcatcactaccagatcgaacttactgttcagattagtctacataattggtaatccagatacacctttaagcacttcaacaggggcaataatatcattgttgacattatttgttgaatctccaggtcaattaattcaaagaatcgctgatgatcctgatgctgtttttaaattagtagaggtggttcctgaggttggtaatcctggagaattaacttttgcatctagaggaattaacttggataaacaagctcaacaatactttagattggctgagaaaaatgatcaaggatattatgtaagtttggggtttgaaaatccaccaaatgatgatgatataacgtcaagtcctgaaatcttaaattatattttagcatctgtacttgcacagatctggattctcctagctaaggctgtaactgctccagacacaggtggtgaggctgaaaatcgtaggtggattaaattgatgcaacaacgcagagtggatggtgagcttagattaagtaaaggatggttggacttagtgaggaataaaatcgcatcggatatcacaattagaaggtttatggtagcattagttcttgacattaaacgttctcctggaacaagaccaagaattgctgaaatgatttgtgatatagacaattatattgtggaggccggactggcaagttttctgttaactatcaaatttggtatagaaacacgttacccagcattggcgttacatgagttttcgggggaattagccactattgaaggactcatgaaattgtaccagtctatgggagaaatggcaccatacatggtcattctagagaattcgatccagactaggtttagtgctgggtcttatccgttactctggagctatgctatgggtgttggtgtagaacttgagagatcaatgagtggattaaacttcacaagaagtttctttgatcctacgtacttcaggttgggtcaggagatggtaagaaggtcttcaggaatggttaatagctcatttgctaaagaacttggactatctgaacatgaaacacaacttgttagccagatcattaactctggtggtgaatcaggtataccgaaatttgatggatttagagcaaacccaacaacatttctaggggctaaggacaacatcactgataggagtgaagatccattgattgcaattccagggtcatcaggacaaccattgccaggtcatgaccccaatatctcaggtgactcatatagaattgatagtagcactaaagacacgaacaatatatcagatggaggaacaaatccaagtcatgatgtttccaattctgctatggaagagctgagaagattggtagagtctaccaacaagattgatacaaagaaatctgaaagcccaggcattgttaatcattacaacgatactgaccttctgagataataaggatatattcaggtagatctttacagaatttaaattaagaaaaacttaggacctcaaggttcacactcctctggccttcatcagaactcggccaattcctcactcactccatgtcagcagaacaaatccaacaagttagacatggccttgaatccttgcaagagatcaaaaacaaccctccaccctctcaagatgtcaatcttgccagggaaatttacgaatccattaaacaaacaggaacaccttcaacacaaggagggaccattacaggaaataatactacgtcagggtgtgacaattactcaatgcatagccagggatcaggtccttctgtttcaggtgctgacaagaatatcgagagacttactggacccgattattcagaattatgggatccagaaggtaacctctgcatgctattcgaaagcgatgatgatgacaacaattattcagagattaatggccggtctaccgctatcgaaggattggatgaacagaataataaggacccaggtattaaacaatcaggagatcagtgttctgaaggagtgtctaagattaattcatcttctagtccccaagaagctacattatcttctgggagatctgatatatctgggacaggagtatctccctgtgcctctttggatataactgttaatgaattagaagatgcaactgttaagaatagtaataatatgaaaggaaattggccaatcccaaagttgcttgtcaaaccaccaccaagaatgaaatcactttctgactctgttacaccattaaaaggggccaccgacgggaaatcagtcttacctgggatggagattacattgtccgggaagaatggtgcaaccctacctgtacacccatttacacaacctgtaaaagactcaaatgcagatgtaagcaatgtccgtcaacatgtcccaagtgtgactgatggttatagtgatgataatgaggaagtacccggtttgcataaagaaactatagacaaagctgatctatctatgcaggacatatacaatttaattcttggatttaaggatgattacaggaaactatcaaataaattggatatgatactagagatgaaacaagatattgataatcttaaaaagagtagtgcaaaaatacaacttgcattatcaacaattgaaggacatctgtccagtgttatgattgctattccaggttcaggtattgatatgaatcaagatgagaagaaggatcaattaaactctgacttaaagccattactagggagggaccattgccgtgcatttcgtgaagtcactaatcctttagatgaaacgtcattgaccaacgctccgaccaaacatgttgctaagatcaacaaaaattgcactcttcagaaaatcaataagaatgagacatctgcaattaagtttgtacctaatgatagctatgcaagtatctcgactatcaagtctattgtcaaatcctcaaaccttaatcaagagcttaaagtcaagttactgacaattctatctcaaattaaaggggtagacaatattaaggagttttatgagaaagttatgatattgatcaagaataataactgatcttgactaatcaatagatactacttatcaaatctagctctgacatcaagtgaattcatctttattaacaagtattaatcttaaataattataaaaaacttaggagttcaggatcagtgggtcatatacaatatgactgagatattcaatctggatgaaagttcatggtcagtcaagggaacactggacccattgacgcctgatacttatcctgatgggcgcctagtacccaagattcgggttattgatcccggtctaggtgatcgtaaaagtggaggatatatgtacttactccttcacggtgtcatcgaggacagtgagaccgtcataaatccgaaagggagagcatttggagctttccctttaggtgtagggcaatcaaccgagaacccagaagacttatttaaggaaatattaaccctcaacattgttactcgcaggactgctggcttcaatgaaaaattggtgtattataatactacacctctaaatctactaaccccttggaaaaaagtactagcatatggaagtatctttactgctaatcaggtctgcaataatacaagttctatccctatagacattcctcagaaatttcgacctgtctatttaactgttaccaagttatcggatgatggatattatcagatacctaaaatgatacaggatttcaaatcatcaaactctgttgcatttaacatccttgtgcatctatcaatgggaacaattttacttgactcatctaaaggctctcgagtaggaaatcctgcagaaaatttgatcacattcatgattcatattgggaatttcaaacggaagaataataaagcttattctcccgaatattgtaagaggaaaataatgaggcttggattaatcttctcactaggagccattggtggaacaagtttgcatattcgatgcacaggcaaaatgagtaagcgattacaagcctacttagggtttaaaagaactttatgttatcctctgatgtatgtcaatgagggtctaaacaaaaccttatggagaaatgaatgcagaattgagaaggttcaagcagtattacagccatcagttccgaatgaatttaagatttatgatgatataatcattgataacacgaatggcctctttaaggttaagtaagctgtgactagtatcaggagttactagtcaaaatcatgtgttgatatccgaattaatagctttaagttgaatatattaaacctgtgataattcaaatttgaaacataattagtatgtagtattgtattaatcagtttgtaatcttgtttgaggatccaaattataacctattaggtattgccactccagcttacaggtaaatctaagcgaatatacaaataattgatattcgggattaaacaatacttgcatattaatccataggtatattagattttactatattcaattattataatgtttattgagttaagctctcatgattataaaaaacttaggattccacataatcacagtttgattgccaattgatgtgtttagtattagttgtgtgaaatattgatattaataaggttaatcaacttttgtacagaagtgaaggtgtaattagatagaaatagattaatccttagtagccgttttgataattgaattgattcttgttttaattctgaattgagattattaatcaccagctcggcataatgtataagattaaggttgtaatcatgggttttttactgttatcagatattacatttgcacaggtaggttgggataatttaacctcaattggagttataagtactaaacaatataactataagataactactttgaatactaatcaactcatggtgattaaaatggtacccaatatatcatcaattattaactgtactaaacttgaattagcaaaatatagggaactgattacaggaatactgagaccaattaatgaatcattagaattgatgaattcatatatcaacatgagaacaggttcagagagattcataggggctgttatagcaggagtagctctaggggttgcaactgcggcgcagataacatcgggaattgccttacataattcgattatgaataaaaaacagatacaggaattaaggaaagcccttagtactacaaataaggcaattgatgagataaggattgcaggtgaaagaactctgatagctgtccaaggtgtgcaagattacattaacaatgttattatccctatgcaagagaaactccagtgcgatattttagcctcacagctatctattgccctactcagatactatactaatatactgactgtttttggaccaagtataagagatcctattactagtacaatttctatacaagctctcagtcaagcattcaatggtaatctacaggcattgcttgatggattagggtatactggacaagacttacatgatctcatagaaagtagatctatcactggtcaaataattcacgctgatatgactgatttattccttatattgagaatcaattatccatctattacggatatgcaaggagtggtaatatatgagctgaattctatcacatatcatattggacctgaagagtggtacactattatgcctaatttcatagctgttcagggatttctggtatctaatttcgatgaacgtaaatgttcaattactaaaacaagtatactgtgtcaacagaattcaatttatcctatgtcaaccgaaatgcaaagatgtataaaaggtgagattaaattctgtccaaggtccaaagcaattgggacattagttaatcgatttatattaattaatgggaatctaatggccaattgtttgggtattatttgtagatgttatacctcaggtcaaattataacgcaagacccaaataaattaatcacaattatatcacaagaagaatgtagagaggttggtgttgatgggattcgtataatggtgggacctaaaaaattaccggatgttatctttaatgccagactagaaataggtgtacctatctcattaagcaagctggatgttgggaccgatttggcaattgcttcagctaaactcaataactctaaggcacttttggagcagtctgataaaatcttaaattctatgtctaagttggattctttaaattcacgtatcttaggatctgtctttataatgatgataatctttgtgattgtaattgtgattatttggattatttgtaagaagtgtagaaataagaggaacaaattaagtgcttctattgaacccctctacatacctccctcttataattcaccccatagcatagttaaatctatttgaaatataagtgtataatctgatataacagatgcagtagaattattaatcaatgataatattattatgataatgattcagttagatgttcattatatctcataacttaatattgacaaatttcaattagttaaatttattctcttcataatatgtatttgtttaattatcctagattaatgtattgttattaaactggtcatctttaatacctaactcagcaatactatcctatacacatgtattagctaataacgatgtaatattgccatttaataataagtacctagtagaatgggaagcattagctgtagtcaatgaatcattatctgctcaattagaaaaaayttaggaatccatgttaatgggagttggccatcatggagtctaataacaacaagtactataaagattcaaaccggtattttagcaagatactagatgagaacaagacggtaaataatcatctgtatagtcttagtataaggataattaccgttatagctattgttgtgagtctaattgcaacaacaataaccatcattaatgctataagcggaaggactactcttaataataatatggacatgctactcaaccaacaagacaagattaataatatcaaggaaatgatatttgatcgtatctatcccctgataaatgccatgagtacagagcttggtcttcacattccaactttattggatgagctgactaaatcaattgatcaaaaaatcaagataatgactccaccacttgaaactacgacatctaatctcaattggtgtatcaaccccccaaatggcattattgtagatcctaaaggttactgtgaaggcttggaactgtcaaaaacttataagttattacttgatcaattagatatgttaagaaagaaatcacttattattaataagaaaagtattaatcagtgtagacttgttgatagctcgaatatcatctttgcaacagttaatatacaatctacaccgagattcttaaatcttggtcacacagttagtaaccaacgtataacattcggtcaaggaacatatagtagcacttatattataactatacaagaggatggattaactgatgttcagtaccgagtatttgaaataggatatatctcagatcaatttggaaccttcccttctctaatcgtttctagagtactacctgtgcgaatggtacttggaatggaatcttgtacactgaccagtgacaagttcgggggttattttttatgcatgaacattccgacacgctctatatatgattatgtcaacataagagacttaaagtcactatacgtcacaatccctcattatggcaaaattaattacacttactttaattttggaaaagtcagaagcccacatgaaattgataagatttggcttacatcagaaaggggacagatgatttcaggttactttgcagcatttgttacgattacaattagaaattataacaattatccctataaatgcttacataacccgtgtcttgaaagatctgagagttattgcaaaggatggtacaaaaatattacaggtactgatgatgttccaatattagcatatctattagttgaaatgaaggatgaggaaggacctttaattacactggttgaaataccaccttacaattatacggctccttctcataattccctttactatgatgataaaattaacaaattaataatgacaacatctcatataggatacattcaaatcaatgaagtgcatgaagtcattgtcggggataatcttaaggctattctcttaaacagattatctgatgaacaccctactcttactgcttgtagatttaatcaggaaattaaagagcgacatatatctgatgggttaataatatctaactctgctcttattgatatacaagaacgtatgtatattacagttaaggctgttccacccataggaaattataacttcacggtagagttgcattcacggtcaaatacatcttacgtagggttgccaaggcagttcaatgctaggtatgacaaactgcatctcgaatgctttgcctgggataggtcttggtggtgcgctttgatacctcaattttcattaagttggaatgaatctctttcagtagatactgccattttcaacttaataaactgtaattaagtttgtggcttgttctagattgatcatttgaataacagttgattaagccgaagttagtaaatacatacattaacctgttcttgaccaagtatgtatcctaatccaattataaaaaacttaggactcaaggtgttgatggcaatggagcaatcagattatcaagatattttatatccagaggtacatctcaacagtcctatagttatctctaaattagtgggtattttggagtattctaaggttgttcacaatcagcagttatctgatcacacaatagtcaagaatatacaatttagattgagaaatggattcaatagtccaagagtacaaacactgttagttatgggtgaaattatcaataaaatcaaaaataaatacccaaattatttgcacataccttatcctgaatgtaatcaaaagttatttaggatggctgacccggagttaacatctaaactagaagccctcttggacaaaggtgacacattatatcttaagattaagacagagatcatagcttgtttcgataagttaaaaactaaaatgagcataaccaatgatctgattagtgacaataggcagctaatttcagatctacctctaattgtcaagggatctcaatggtttttcccttttttgctctggttttctgttaaaactgagactaggaactgtattcgacaaaatcaaaaaactcgtgttaggtcacaataccgacctcatttgtcagaaactaaaagaattacgctggtcgttacccctgacttgatcacaatatttgaccacgtcaacaaatgtatatatcatctgacttttgagatgttgttgatgtattgtgatgtagtagaagggaggttaatgaccgaagcatctatgagtctagatcacagatttattaacctattgtcgagggtccagtatatgtgggatctattagatgggatgtttgagagtctaggaaatcagctatattcaatcattgcactcttagaacctctctctcttgcctatctacagttgatggatgcagacccacagatacggggtacatttttacaccattgcctttcagagttggaagaactcttatttagtaaatccccttttgatcctgtgatttatgaaaatctaattagtggacttgattacatctatttaacagacgatattcatttaactgctgagatattttctttctttagaagttttggtcatccttatttagaagcacaaaatgcagctagcaatgttaggaaatatatgaatcaacctaaagttatctcataccagactctaatgcaaggacatgcaattttttgtggcattataataaatgggttcagagatcgtcacggagggacatggccacctgtagagctaccacatcatgcatccgctgtaattagaaatgctcagttatctggagaaggattaacacctgagcagtgtgctcaatactggaggtcattttgtggatttaaatttaaatgttttatgccattaagtctagatagcgacctcaccatgtaccttagagataaggcattatcacctattaagaatgagtgggattctgtgtatgctaaagagtatttaagatacaaccctggcttaccgactagctctcgaagattagtcaatgtatttctagaagatgataaatttgatccgtacgaaatgattatgtacgtaataaacggtgattatttaagggataatgagttcaatctctcatatagtcttaaagaaaaggagatcaaggaggtaggccgattgttcgctaaaatgacttataagatgagagcttgtcaggtaatagcagaaaatttaattgcaaatggagttgggaaattttttaaagacaatgggatggcgaaggatgaacataaattaaccaaaacattacataagctggctatttctggtgtacctaaagataattctcaactctatttaagtgaatgttgggaacaagtggtagaacaatgcgtaaccagtacgcaaacaaaaaatcaaattatcagttcacactcaggaaaatcagttgcatcaaagttttcaagatcaaatcccaatgataggggtattctaaatagtggtagacatttgaataaacatccaaaacatccatcaaacaccgaatactatgaaactgtcagtagttttataactactgatctcaagaaatattgcctcaactggcgctatgaatcaagtagtgtgtttgcagaaagactcaatgagatttatgggttaccaggatttttccattggcttcatagaattttggagaaatctgtattatatgttagtgatccatccagtccacctgattttgatcaacatgtcgatattgattcagttccaaatgatcatatttttatcaaatacccaatgggtgggataaaaggattttgtcaaaaattatggacaatcagcacaatcccatttttatatttagcagcctttgatacaggggttagaatatcttcgttggttcaaggtgataatcaagcaattgcagtgaccaaaagagttccatcatcctggagttattcgagaaaaaaagaggagtcaactaaagttacaacacaatattttttaaacttgagacaacgcttacatgatataggtcatgagttaaaggcaaatgagactattatatcttcacacttttttgtttactctaagggtatttattatgatggtatacttctttcacaatcccttaaaagtattgcaagatgtgttttttggtccgagacaattgtcgatgagactaggtcagcttgcagcaatatatccactacccttgctaaagctattgaacggggttatgataaatttgtagcatacgctattaatatatataagactatacaccaggtcttaattgcattatcttttactattaatcccactatgactccggacataacagaacctttttataaaagtttagatttacttaaaaacctcattctgataccagcaccattgggtgggatgaattacatgaatatgagcagattatttgttaggaacataggtgatcccattacagcttcatttgctgacatcaagcgtatgatcgaatgcgggttattagggcacaatgttctctcacaaataatgtatcagaaatgtggtacctcgaaatacttagattgggctagtgacccttattccataaatcttccttatagtcaaagcatgaccaaagtattaaaaaatataaccgcgagatatgttctcatgcatagtcctaaccctatgctaaaagatttattccatgagaagtcacaagaagaggatgagattcttgctgaatttttgctggatcgtcagttaataatccctagagctgcacatgaaattttatcgaattcagtaacaggagctagagagtcgattgcagggatgcttgatactactaaaggacttattcgagccagtatgtcaagaggtggtctgacatcttcacttgttttgaaattgtcaacatatgattatcaacaatttagaacatgccttgaatggctttatgcccctaccacaggaatagcagtaagtgctgattcttgttcagtttttttagccagagctattcgaaaaaggatgtgggttcacctgactaaaggaagagaaatttatggcctagaagtgcctgatatattagaatgtatgcagagcaatgtaattgttgatcatgaagattgttattcatgtattcaaggatcaagatactacacatggttttttgtaccttctaattgtcagcttgatcagattaacaagtctacaaattctctacgggttccttacattggctctactacagaggaaagaagtgacatgaaattatcatacgtcagatcccctagtaggccacttaaggcagcagtccgaattgcagcagtctacacatgggcatacggtgatgacgatctgtcttggcgtgaggcttggtacttggcaaggactagggcaaatgttactttcgatgagcttaaattagtaacacccatagctacctctactaacttggcacatagattaagggacaggagtactcaagttaagtattcaggaacttcattggtaagagtggcacgctatacaacaatatccaatgataatatgtcatttgttattaatgacaaaaaggtagatactaattttgtctatcaacagggcatgttattgggtttgagtatcctagaatatatatttagatactgtaaaagtactggtcaatcaaatactgtagttcacttgcatgcagatgttaattgttgcataatccaaatgacagatcaaccttatactccaagcttaacgaaaaaattacctgagattaaacctattaataataaattgatttatgatccagctcctataattgatactgatgcagctaggttatattctcagaagtacttatcacacctgatagattttccaaattggtcaatgaatcagctaaatgtagttttagcaaaagtagttgcaatatctattgtggacttgataactaaagcgagtaaagatcatctcaatgaaattatggcagttgttggagatgatgacattaatagctttataacagaatttttgctagttgatccgaggctatttacattgtacttaggtcaatacacgtcacttcaatgggcatatgaaattcattatcaccgacccgtaggcaaataccagatggcagaagtgttacacactttactgtcaagagcaagtaaaggtatatttaatatattgactaatgcctttagtcatcctagagtttacaaaagattttgggaatgtggattactggagcctatttatggaccatacatagggagccaaaatttatatagtacagtaattgattacctttacaatgcttatataacttatttagatgcttatctatctgatcatatcgaagatgcagacatagtaatatgtgagacagaagaaacttgtctagctaataggattgataactatcaaggtaggcatctcgccgtacttattgatctttattgtgattctactaggtgtcctaatataaaagggtcagacacaatcatgcgaaactcaattctcaaatcttttattgataatgagagaaggacaagtccattaggtctaacatggaatcttgatccattactcatagatcatttcagttgttcaattacttatctgaggagaggtattattaaacagattaggctaaggtttgatccaaacatatctattgagttggttaaattggcaaaacctgaagtgattcatcaaggaccaaaaataccgtcttcttgggcccttatagatattaatcctgaggtcaatgatcttaatacagttttcggagaattaaatagtaaatggaaagatattcctattggacaaattagaattcaaaattttgagatccatgcttaccgaagaattggagttaattcaactgcatgttataaagcattggaaatgctatctgtactaactcggtttatgtctaacccagcaggagctttgtttttaggagagggtgcagggtcaatgttagttacctatcgtgcgtttatcccgttcaagagaatttattataatagtggagtttctatacaaaatattcaaagccaaagggaactaagtctatacccatctgaagtagccttggtcgataataaaaatcgtttgaccagtgatcctgatatcaaagtcttatttaatggcaagccagaatccacgtgggttgggaatatagactgctttgcttatattctgagtcatattgaaacttctagtttaacattaatccacagtgatattgaatctagcttgagtaaaacaaagaataagattcttgaggagctttgccatattctatcaatggcactgattctaggaaagattggatctgtattagttattaagctattaccacgggttggtgactacacatattcattttgcaagtatgcgtcagaattctaccaacagaatttcttcattttacctagatttagtaacatgtcatcatctgaaatttactacgttggagttcatttaaataccaatagactggttgatccagataggattgtgcaatatataatcaggaatctccaatctactccagtcactttcttatcttacattttggaaactaaatatagaaataatatggttacaaattatgggctctgtttgtctgatggacataaaagcgattacttgtcatcaatcaccaagatagaaaatgttcttttatcatgtggattggaattgaatggacctaagattattcagcaattatctggacatgactacgccaatggagagattagcttagaatcaagtataatggtactggtcagagaatatctaaatgcaactatccaaggtcgagaaacactaggtcttttttcaccttaccctgtgttacatgagagtcagttaagagaaattaacaggtgcattgcattgaagtatgttgtatatttacttttttactcaacctctgtaggatctagtagacagatcatgagcaatctcagaaaaggagtattaatgtatgacttaagagatgagtttttcatggaaaggttatcaacaaatttcaagaaaaaaataatgtcacaagaggttaaaactacatggatctttaatattgatgtaccaacaagaaaagctctgtataaattagttggttattcacttatcattaatcacgtataacaagtgtattgagttggtaatattctagatgaacaagtataggtttatgtacagtaagtgattaaatattagattcaggtagataaacttcctaatagtgtatcctatagataacctaaggctatttgatgttagattaattagaaaaaacttcttgaattatgatagacttcaacccctggctaagacttatcatttaaaattataaccaagttgtcctgataatatcagatctcattaattacttgatagcgtaatataacaggtgcatgatgatcctttattactcatatacctgttattaagctcctgttcacattatcccctatttaagttgccttttaaattacctaatatgtttagtaatgagaaacattgatacatacaaagctaaagaagcctgattttatctaaggttgtatctaattgttgtcaatttataattcggaatatctgggccctaaacctcctccaaatatactaaaaggttttaaaaaaacaaaaaaggtttcttacttattgtacggacctatagctttcttttgtctggt

SEQ ID NO: 9 - protein, 519 aa, Feline Paramyxovirus-Type 2
  Nucleocapsid protein, Strain TV25
MASLLRSLAAFKKHREQPTVPSGSGGTIKGLKNTIIVPVPGDTVITTRSNLLFRLVYIIGNPDTPLSTSTGAIISLLTLFVESPGQLIQRIADDPDAVFKLVEVVPEVGNPGELTFASRGINLDKQAQQYFRLAEKNDQGYYVSLGFENPPNDDDITSSPEILNYILASVLAQIWILLAKAVTAPDTGGEAENRRWIKLMQQRRVDGELRLSKGWLDLVRNKIASDITIRRFMVALVLDIKRSPGTRPRIAEMICDIDNYIVEAGLASFLLTIKFGIETRYPALALHEFSGELATIEGLMKLYQSMGEMAPYMVILENSIQTRFSAGSYPLLWSYAMGVGVELERSMSGLNFTRSFFDPTYFRLGQEMVRRSSGMVNSSFAKELGLSEHETQLVSQIINSGGESGIPKFDGFRANPTTFLGAKDNITDRSEDPLIAIPGSSGQPLPGHDPNISGDSYRIDSSTKDTNNISDGGTNPSHDVSNSAMEELRRLVESTNKIDTKKSESPGIVNHYNDTDLLR

SEQ ID NO: 10 - protein, 491 aa, Feline Paramyxovirus-Type 2
  Phosphoprotein, Strain TV25
MSAEQIQQVRHGLESLQEIKNNPPPSQDVNLAREIYESIKQTGTPSTQGGTITGNNTTSGCDNYSMHSQGSGPSVSGADKNIERLTGPDYSELWDPEGNLCMLFESDDDDNNYSEINGRSTAIEGLDEQNNKDPGIKQSGDQCSEGVSKINSSSSPQEATLSSGRSDISGTGVSPCASLDITVNELEDATVKNSNNMKGNWPIPKLLVKPPPRMKSLSDSVTPLKGATDGKSVLPGMEITLSGKNGATLPVHPFTQPVKDSNADVSNVRQHVPSVTDGYSDDNEEVPGLHKETIDKADLSMQDIYNLILGFKDDYRKLSNKLDMILEMKQDIDNLKKSSAKIQLALSTIEGHLSSVMIAIPGSGIDMNQDEKKDQLNSDLKPLLGRDHCRAFREVTNPLDETSLTNAPTKHVAKINKNCTLQKINKNETSAIKFVPNDSYASISTIKSIVKSSNLNQELKVKLLTILSQIKGVDNIKEFYEKVMILIKNNN

SEQ ID NO: 11 - protein, 337 aa, Feline Paramyxovirus-Type 2
  Matrix protein, Strain TV25
MTEIFNLDESSWSVKGTLDPLTPDTYPDGRLVPKIRVIDPGLGDRKSGGYMYLLLHGVIEDSETVINPKGRAFGAFPLGVGQSTENPEDLFKEILTLNIVTRRTAGFNEKLVYYNTTPLNLLTPWKKVLAYGSIFTANQVCNNTSSIPIDIPQKFRPVYLTVTKLSDDGYYQIPKMIQDFKSSNSVAFNILVHLSMGTILLDSSKGSRVGNPAENLITFMIHIGNFKRKNNKAYSPEYCKRKIMRLGLIFSLGAIGGTSLHIRCTGKMSKRLQAYLGFKRTLCYPLMYVNEGLNKTLWRNECRIEKVQAVLQPSVPNEFKIYDDIIIDNTNGLFKVK

SEQ ID NO: 12 - protein, 543 aa, Feline Paramyxovirus-Type 2
  Fusion protein, Strain TV25
MYKIKVVIMGFLLLSDITFAQVGWDNLTSIGVISTKQYNYKITTLNTNQLMVIKMVPNISSIINCTKLELAKYRELITGILRPINESLELMNSYINMRTGSERFIGAVIAGVALGVATAAQITSGIALHNSIMNKKQIQELRKALSTTNKAIDEIRIAGERTLIAVQGVQDYINNVIIPMQEKLQCDILASQLSIALLRYYTNILTVFGPSIRDPITSTISIQALSQAFNGNLQALLDGLGYTGQDLHDLIESRSITGQIIHADMTDLFLILRINYPSITDMQGVVIYELNSITYHIGPEEWYTIMPNFIAVQGFLVSNFDERKCSITKTSILCQQNSIYPMSTEMQRCIKGEIKFCPRSKAIGTLVNRFILINGNLMANCLGIICRCYTSGQIITQDPNKLITIISQEECREVGVDGIRIMVGPKKLPDVIFNARLEIGVPISLSKLDVGTDLAIASAKLNNSKALLEQSDKILNSMSKLDSLNSRILGSVFIMMIIFVIVIVIIWIICKKCRNKRNKLSASIEPLYIPPSYNSPHSIVKSI

SEQ ID NO: 13 - protein, 595 aa, Feline Paramyxovirus-Type 2
  Hemagglutinin, Strain TV25
MESNNNKYYKDSNRYFSKILDENKTVNNHLYSLSIRIITVIAIVVSLIATTITIINAISGRTTLNNNMDMLLNQQDKINNIKEMIFDRIYPLINAMSTELGLHIPTLLDELTKSIDQKIKIMTPPLETTTSNLNWCINPPNGIIVDPKGYCEGLELSKTYKLLLDQLDMLRKKSLIINKKSINQCRLVDSSNIIFATVNIQSTPRFLNLGHTVSNQRITFGQGTYSSTYIITIQEDGLTDVQYRVFEIGYISDQFGTFPSLIVSRVLPVRMVLGMESCTLTSDKFGGYFLCMNIPTRSIYDYVNIRDLKSLYVTIPHYGKINYTYFNFGKVRSPHEIDKIWLTSERGQMISGYFAAFVTITIRNYNNYPYKCLHNPCLERSESYCKGWYKNITGTDDVPILAYLLVEMKDEEGPLITLVEIPPYNYTAPSHNSLYYDDKINKLIMTTSHIGYIQINEVHEVIVGDNLKAILLNRLSDEHPTLTACRFNQEIKERHISDGLIISNSALIDIQERMYITVKAVPPIGNYNFTVELHSRSNTSYVGLPRQFNARYDKLHLECFAWDRSWWCALIPQFSLSWNESLSVDTAIFNLINCN

SEQ ID NO: 14 - protein, 2202 aa, Feline Paramyxovirus-Type 2
  Polymerase, Strain TV25
MEQSDYQDILYPEVHLNSPIVISKLVGILEYSKVVHNQQLSDHTIVKNIQFRLRNGFNSPRVQTLLVMGEIINKIKNKYPNYLHIPYPECNQKLFRMADPELTSKLEALLDKGDTLYLKIKTEIIACFDKLKTKMSITNDLISDNRQLISDLPLIVKGSQWFFPFLLWFSVKTETRNCIRQNQKTRVRSQYRPHLSETKRITLVVTPDLITIFDHVNKCIYHLTFEMLLMYCDVVEGRLMTEASMSLDHRFINLLSRVQYMWDLLDGMFESLGNQLYSIIALLEPLSLAYLQLMDADPQIRGTFLHHCLSELEELLFSKSPFDPVIYENLISGLDYIYLTDDIHLTAEIFSFFRSFGHPYLEAQNAASNVRKYMNQPKVISYQTLMQGHAIFCGIIINGFRDRHGGTWPPVELPHHASAVIRNAQLSGEGLTPEQCAQYWRSFCGFKFKCFMPLSLDSDLTMYLRDKALSPIKNEWDSVYAKEYLRYNPGLPTSSRRLVNVFLEDDKFDPYEMIMYVINGDYLRDNEFNLSYSLKEKEIKEVGRLFAKMTYKMRACQVIAENLIANGVGKFFKDNGMAKDEHKLTKTLHKLAISGVPKDNSQLYLSECWEQVVEQCVTSTQTKNQIISSHSGKSVASKFSRSNPNDRGILNSGRHLNKHPKHPSNTEYYETVSSFITTDLKKYCLNWRYESSSVFAERLNEIYGLPGFFHWLHRILEKSVLYVSDPSSPPDFDQHVDIDSVPNDHIFIKYPMGGIKGFCQKLWTISTIPFLYLAAFDTGVRISSLVQGDNQAIAVTKRVPSSWSYSRKKEESTKVTTQYFLNLRQRLHDIGHELKANETIISSHFFVYSKGIYYDGILLSQSLKSIARCVFWSETIVDETRSACSNISTTLAKAIERGYDKFVAYAINIYKTIHQVLIALSFTINPTMTPDITEPFYKSLDLLKNLILIPAPLGGMNYMNMSRLFVRNIGDPITASFADIKRMIECGLLGHNVLSQIMYQKCGTSKYLDWASDPYSINLPYSQSMTKVLKNITARYVLMHSPNPMLKDLFHEKSQEEDEILAEFLLDRQLIIPRAAHEILSNSVTGARESIAGMLDTTKGLIRASMSRGGLTSSLVLKLSTYDYQQFRTCLEWLYAPTTGIAVSADSCSVFLARAIRKRMWVHLTKGREIYGLEVPDILECMQSNVIVDHEDCYSCIQGSRYYTWFFVPSNCQLDQINKSTNSLRVPYIGSTTEERSDMKLSYVRSPSRPLKAAVRIAAVYTWAYGDDDLSWREAWYLARTRANVTFDELKLVTPIATSTNLAHRLRDRSTQVKYSGTSLVRVARYTTISNDNMSFVINDKKVDTNFVYQQGMLLGLSILEYIFRYCKSTGQSNTVVHLHADVNCCIIQMTDQPYTPSLTKKLPEIKPINNKLIYDPAPIIDTDAARLYSQKYLSHLIDFPNWSMNQLNVVLAKVVAISIVDLITKASKDHLNEIMAVVGDDDINSFITEFLLVDPRLFTLYLGQYTSLQWAYEIHYHRPVGKYQMAEVLHTLLSRASKGIFNILTNAFSHPRVYKRFWECGLLEPIYGPYIGSQNLYSTVIDYLYNAYITYLDAYLSDHIEDADIVICETEETCLANRIDNYQGRHLAVLIDLYCDSTRCPNIKGSDTIMRNSILKSFIDNERRTSPLGLTWNLDPLLIDHFSCSITYLRRGIIKQIRLRFDPNISIELVKLAKPEVIHQGPKIPSSWALIDINPEVNDLNTVFGELNSKWKDIPIGQIRIQNFEIHAYRRIGVNSTACYKALEMLSVLTRFMSNPAGALFLGEGAGSMLVTYRAFIPFKRIYYNSGVSIQNIQSQRELSLYPSEVALVDNKNRLTSDPDIKVLFNGKPESTWVGNIDCFAYILSHIETSSLTLIHSDIESSLSKTKNKILEELCHILSMALILGKIGSVLVIKLLPRVGDYTYSFCKYASEFYQQNFFILPRFSNMSSSEIYYVGVHLNTNRLVDPDRIVQYIIRNLQSTPVTFLSYILETKYRNNMVTNYGLCLSDGHKSDYLSSITKIENVLLSCGLELNGPKIIQQLSGHDYANGEISLESSIMVLVREYLNATIQGRETLGLFSPYPVLHESQLREINRCIALKYVVYLLFYSTSVGSSRQIMSNLRKGVLMYDLRDEFFMERLSTNFKKKIMSQEVKTTWIFNIDVPTRKALYKLVGYSLIINHV